European Patent Application EP 4 534 547 A1, published April 9, 2025. Title: 親和性物質、化合物、抗体およびそれらの塩. Applicant: Ajinomoto Co., Inc. The sequence listing filed with the application follows.

SEQUENCE LISTING (79 sequences)

SEQ ID NO: 1 - protein, 90 aa, synthetic construct
  REGION 1..90: note = Affinity polypeptide (QET-Z34CM-PA32-Fc3K).The N-terminal andC-terminal amino acid residues may be protected.
QETFNMQCQRRFYEALHDPNLNEEQRNARIRSIREECGGAAPAAPAPAAPAAPAPAAPAAPAPAAPAAPAPGGRGNCAYHKGQIIWCTYH

SEQ ID NO: 2 - protein, 106 aa, synthetic construct
  REGION 1..106: note = Affinity polypeptide (QET-Z34CM-PA48-Fc3K).The N-terminal andC-terminal amino acid residues may be protected.
QETFNMQCQRRFYEALHDPNLNEEQRNARIRSIREECGGAAPAAPAPAAPAAPAPAAPAAPAPAAPAAPAPAAPAAPAPAAPAAPAPGGRGNCAYHKGQIIWCTYH

SEQ ID NO: 3 - protein, 90 aa, synthetic construct
  REGION 1..90: note = Affinity polypeptide (QET-Fc3K-PA32-Z34CM).The N-terminal andC-terminal amino acid residues may be protected.
QETRGNCAYHKGQIIWCTYHGGAAPAAPAPAAPAAPAPAAPAAPAPAAPAAPAPGGFNMQCQRRFYEALHDPNLNEEQRNARIRSIREEC

SEQ ID NO: 4 - protein, 106 aa, synthetic construct
  REGION 1..106: note = Affinity polypeptide (QET-Fc3K-PA48-Z34CM).The N-terminal andC-terminal amino acid residues may be protected.
QETRGNCAYHKGQIIWCTYHGGAAPAAPAPAAPAAPAPAAPAAPAPAAPAAPAPAAPAAPAPAAPAAPAPGGFNMQCQRRFYEALHDPNLNEEQRNARIRSIREEC

SEQ ID NO: 5 - protein, 100 aa, synthetic construct
  REGION 1..100: note = Affinity polypeptide (QET-Fc3K-PA32-ProAR).The N-terminal andC-terminal amino acid residues may be protected.
QETRGNCAYHKGQIIWCTYHGGAAPAAPAPAAPAAPAPAAPAAPAPAAPAAPAPGGFNREQQNAFYEILHLPNLNEEQRNGFIQSLRDDPSQSANLLAEA

SEQ ID NO: 6 - protein, 116 aa, synthetic construct
  REGION 1..116: note = Affinity polypeptide (QET-Fc3K-PA48-ProAR).The N-terminal andC-terminal amino acid residues may be protected.
QETRGNCAYHKGQIIWCTYHGGAAPAAPAPAAPAAPAPAAPAAPAPAAPAAPAPAAPAAPAPAAPAAPAPGGFNREQQNAFYEILHLPNLNEEQRNGFIQSLRDDPSQSANLLAEA

SEQ ID NO: 7 - protein, 117 aa, synthetic construct
  REGION 1..117: note = Affinity polypeptide (QET-ProAR-PA32-Z34CK).The N-terminal andC-terminal amino acid residues may be protected.
QETFNREQQNAFYEILHLPNLNEEQRNGFIQSLRDDPSQSANLLAEAGGAAPAAPAPAAPAAPAPAAPAAPAPAAPAAPAPGGFNKQCQRRFYEALHDPNLNEEQRNARIRSIREEC

SEQ ID NO: 8 - protein, 133 aa, synthetic construct
  REGION 1..133: note = Affinity polypeptide (QET-ProAR-PA48-Z34CK).The N-terminal andC-terminal amino acid residues may be protected.
QETFNREQQNAFYEILHLPNLNEEQRNGFIQSLRDDPSQSANLLAEAGGAAPAAPAPAAPAAPAPAAPAAPAPAAPAAPAPAAPAAPAPAAPAAPAPGGFNKQCQRRFYEALHDPNLNEEQRNARIRSIREEC

SEQ ID NO: 9 - DNA, 363 bp, synthetic construct
  misc_feature 1..363: note = Nucleotide sequence of the polynucleotide encoding thepolypeptide CspBss-QET-Z34CM-PA32-Fc3K
  source 1..363: mol_type = other DNA
atgtttaacaaccgtatccgcactgcagctctcgctggtgcaatcgcaatctccaccgcagcttccggcgtagctatcccagcattcgctcaggagaccttcaacatgcagtgccaacggcgcttttacgaagcgctccacgatcccaacctgaacgaggaacagcgtaacgcgcgcattcgctccatccgtgaggaatgtggcggtgctgcccctgctgccccagcaccggcagcacctgcggcaccagctccggcagctccagctgcaccggcccctgccgctccagcagcgccagctcccggaggtcgaggcaattgcgcctatcacaaggggcagatcatctggtgcacttaccattaa

SEQ ID NO: 10 - protein, 120 aa, synthetic construct
  REGION 1..120: note = Amino acid sequence of the polypeptide CspBss-QET-Z34CM-PA32-Fc3K
MFNNRIRTAALAGAIAISTAASGVAIPAFAQETFNMQCQRRFYEALHDPNLNEEQRNARIRSIREECGGAAPAAPAPAAPAAPAPAAPAAPAPAAPAAPAPGGRGNCAYHKGQIIWCTYH

SEQ ID NO: 11 - DNA, 411 bp, synthetic construct
  misc_feature 1..411: note = Nucleotide sequence of the polynucleotide encoding thepolypeptide CspBss-QET-Z34CM-PA48-Fc3K
  source 1..411: mol_type = other DNA
atgtttaacaaccgtatccgcactgcagctctcgctggtgcaatcgcaatctccaccgcagcttccggcgtagctatcccagcattcgctcaggagacctttaacatgcagtgccaacgtcgtttttacgaagcgctgcacgatcccaacctgaacgaggaacagcgcaatgcgcgaatacgctccattcgcgaggaatgtggcggagcagctcccgcggctcctgctccagcagcgcctgctgctcctgcccctgcggcacctgcagcacctgcaccagcagctccggcagcaccagctccagctgcacccgccgccccagctcctgcagcgccagccgctccggcccccggaggtaggggcaactgcgcatatcacaaggggcagataatctggtgcacttatcactaa

SEQ ID NO: 12 - protein, 136 aa, synthetic construct
  REGION 1..136: note = Amino acid sequence of the polypeptide CspBss-QET-Z34CM-PA48-Fc3K
MFNNRIRTAALAGAIAISTAASGVAIPAFAQETFNMQCQRRFYEALHDPNLNEEQRNARIRSIREECGGAAPAAPAPAAPAAPAPAAPAAPAPAAPAAPAPAAPAAPAPAAPAAPAPGGRGNCAYHKGQIIWCTYH

SEQ ID NO: 13 - DNA, 363 bp, synthetic construct
  misc_feature 1..363: note = Nucleotide sequence of the polynucleotide encoding thepolypeptide CspBss-QET-Fc3K-PA32-Z34CM
  source 1..363: mol_type = other DNA
atgtttaacaaccgtatccgcactgcagctctcgctggtgcaatcgcaatctccaccgcagcttccggcgtagctatcccagcattcgctcaggagacccgtggcaactgtgcctaccacaagggccagatcatctggtgcacgtaccacggaggtgccgcgcctgccgcacctgctccagctgctcccgctgcccctgcaccagctgcgccagcagcaccagctccagcggcacctgcagcaccggcacctggtggcttcaacatgcagtgccaacgacgcttctacgaggctctgcacgatccgaacctcaacgaggaacagcgcaatgcccgtattcggtccatcagggaggaatgctaa

SEQ ID NO: 14 - protein, 120 aa, synthetic construct
  REGION 1..120: note = Amino acid sequence of the polypeptide CspBss-QET-Fc3K-PA32-Z34CM
MFNNRIRTAALAGAIAISTAASGVAIPAFAQETRGNCAYHKGQIIWCTYHGGAAPAAPAPAAPAAPAPAAPAAPAPAAPAAPAPGGFNMQCQRRFYEALHDPNLNEEQRNARIRSIREEC

SEQ ID NO: 15 - DNA, 411 bp, synthetic construct
  misc_feature 1..411: note = Nucleotide sequence of the polynucleotide encoding thepolypeptide CspBss-QET-Fc3K-PA48-Z34CM
  source 1..411: mol_type = other DNA
atgtttaacaaccgtatccgcactgcagctctcgctggtgcaatcgcaatctccaccgcagcttccggcgtagctatcccagcattcgctcaggagacccgtggcaattgcgcctatcacaagggtcagatcatttggtgcacctaccatggtggtgcagcaccagctgccccggctccggctgcgcctgctgcacctgcgccagctgcacctgcagcaccggcacctgctgctccagcagcacccgctcctgcagctcccgctgccccagctccagcggcgcctgcggcgccagcacctggagggttcaacatgcagtgccaacgtcgcttttacgaggctttgcatgatcctaacttgaacgaggaacagcggaatgcgcggatacgctccatacgcgaagaatgttaa

SEQ ID NO: 16 - protein, 136 aa, synthetic construct
  REGION 1..136: note = Amino acid sequence of the polypeptide CspBss-QET-Fc3K-PA48-Z34CM
MFNNRIRTAALAGAIAISTAASGVAIPAFAQETRGNCAYHKGQIIWCTYHGGAAPAAPAPAAPAAPAPAAPAAPAPAAPAAPAPAAPAAPAPAAPAAPAPGGFNMQCQRRFYEALHDPNLNEEQRNARIRSIREEC

SEQ ID NO: 17 - DNA, 393 bp, synthetic construct
  misc_feature 1..393: note = Nucleotide sequence of the polynucleotide encoding thepolypeptide CspBss-QET-Fc3K-PA32-ProAR
  source 1..393: mol_type = other DNA
atgtttaacaaccgtatccgcactgcagctctcgctggtgcaatcgcaatctccaccgcagcttccggcgtagctatcccagcattcgctcaggagacccgcggcaactgtgcctaccacaaggggcagatcatctggtgcacctatcacggtggtgcggctccggctgctccagcgccagcagctcccgctgcaccagccccagcggcacctgccgcacctgcacctgcagctccagcggctcccgcaccgggaggctttaaccgcgaacagcagaacgccttctacgagattctccatctgcccaacctcaacgaggagcaacggaatggcttcatccagagcttgcgtgacgatccgtctcaatccgccaatctgcttgcggaagcctaa

SEQ ID NO: 18 - protein, 130 aa, synthetic construct
  REGION 1..130: note = Amino acid sequence of the polypeptide CspBss-QET-Fc3K-PA32-ProAR
MFNNRIRTAALAGAIAISTAASGVAIPAFAQETRGNCAYHKGQIIWCTYHGGAAPAAPAPAAPAAPAPAAPAAPAPAAPAAPAPGGFNREQQNAFYEILHLPNLNEEQRNGFIQSLRDDPSQSANLLAEA

SEQ ID NO: 19 - DNA, 441 bp, synthetic construct
  misc_feature 1..441: note = Nucleotide sequence of the polynucleotide encoding thepolypeptide CspBss-QET-Fc3K-PA48-ProAR
  source 1..441: mol_type = other DNA
atgtttaacaaccgtatccgcactgcagctctcgctggtgcaatcgcaatctccaccgcagcttccggcgtagctatcccagcattcgctcaggagacccgtgggaactgcgcgtaccataagggccagatcatctggtgcacctatcatggcggtgctgcgcctgcagctccggctcctgccgctccagccgcgccagccccagcagctccagcagcacctgcacctgctgcaccagcggctccagctcctgcggcacccgctgcaccggcaccagccgctccggctgccccagctccgggtggctttaaccgcgaacagcagaacgccttctacgagatactccaccttcccaacctgaacgaggagcagcgaaacggcttcatccagtctcttcgcgatgatccatcccagagcgctaacttgcttgcagaagcgtaa

SEQ ID NO: 20 - protein, 146 aa, synthetic construct
  REGION 1..146: note = Amino acid sequence of the polypeptide CspBss-QET-Fc3K-PA32-ProAR
MFNNRIRTAALAGAIAISTAASGVAIPAFAQETRGNCAYHKGQIIWCTYHGGAAPAAPAPAAPAAPAPAAPAAPAPAAPAAPAPAAPAAPAPAAPAAPAPGGFNREQQNAFYEILHLPNLNEEQRNGFIQSLRDDPSQSANLLAEA

SEQ ID NO: 21 - DNA, 444 bp, synthetic construct
  misc_feature 1..444: note = Nucleotide sequence of the polynucleotide encoding thepolypeptide CspBss-QET-ProAR-PA32-Z34CK
  source 1..444: mol_type = other DNA
atgtttaacaaccgtatccgcactgcagctctcgctggtgcaatcgcaatctccaccgcagcttccggcgtagctatcccagcattcgctcaggagacctttaaccgcgaacagcagaacgccttctacgagatcctgcatctccccaatctgaacgaagagcagaggaatggctttatccagagccttcgtgacgatccgtcgcaatctgccaacctgttggcggaagctggaggtgccgcgccagcggcaccagcaccagctgcaccggctgctcccgcacctgccgcaccagccgctcctgccccagcagctccggcagctcctgcacctggtggcttcaacaagcagtgccaacgtcgcttctatgaagcgctacacgatcccaacctcaacgaggaacagcgcaatgcgcgaatccggtccattcgcgaagagtgttaa

SEQ ID NO: 22 - protein, 147 aa, synthetic construct
  REGION 1..147: note = Amino acid sequence of the polypeptideCspBss-QET-ProAR-PA32-Z34CK
MFNNRIRTAALAGAIAISTAASGVAIPAFAQETFNREQQNAFYEILHLPNLNEEQRNGFIQSLRDDPSQSANLLAEAGGAAPAAPAPAAPAAPAPAAPAAPAPAAPAAPAPGGFNKQCQRRFYEALHDPNLNEEQRNARIRSIREEC

SEQ ID NO: 23 - DNA, 492 bp, synthetic construct
  misc_feature 1..492: note = Nucleotide sequence of the polynucleotide encoding thepolypeptide CspBss-QET-ProAR-PA48-Z34CK
  source 1..492: mol_type = other DNA
atgtttaacaaccgtatccgcactgcagctctcgctggtgcaatcgcaatctccaccgcagcttccggcgtagctatcccagcattcgctcaggagacctttaaccgcgaacagcagaacgccttctacgagatcctccatctgccaaacctgaacgaagaacagcgcaacggctttatccagtccctcagggacgatccgtctcagtcggccaatttgctagccgaagcgggaggtgctgctccggcagcacccgcaccagccgcgcccgctgctccagcgccggcagctcctgcggcaccagctccagcagcaccagcggctccagcacctgccgcacctgcagctccggctcctgcagcccccgccgctcctgcgccgggtggcttcaacaagcagtgccaacgacgcttctatgaggcgcttcacgatcccaacctgaatgaggagcaacggaatgcccgtatccgtagcattcgcgaagaatgttaa

SEQ ID NO: 24 - protein, 163 aa, synthetic construct
  REGION 1..163: note = Amino acid sequence of the polypeptideCspBss-QET-ProAR-PA48-Z34CK
MFNNRIRTAALAGAIAISTAASGVAIPAFAQETFNREQQNAFYEILHLPNLNEEQRNGFIQSLRDDPSQSANLLAEAGGAAPAAPAPAAPAAPAPAAPAAPAPAAPAAPAPAAPAAPAPAAPAAPAPGGFNKQCQRRFYEALHDPNLNEEQRNARIRSIREEC

SEQ ID NO: 25 - protein, 33 aa, synthetic construct
  REGION 1..33: note = Amino acid sequence of peptide fragment
THTCPPCPAPELLGGPSVFLFPPKPKDTLMISR

SEQ ID NO: 26 - protein, 17 aa, synthetic construct
  REGION 1..17: note = Affinity peptide.Two cysteine residues may be linked viadisulfide bridge.
RGNCAYHKGQIIWCTYH

SEQ ID NO: 27 - protein, 12 aa, synthetic construct
  REGION 1..12: note = Affinity peptide
EPIHRSTLTALL

SEQ ID NO: 28 - protein, 10 aa, synthetic construct
  REGION 1..10: note = Affinity peptide
FARLVSSIRY

SEQ ID NO: 29 - protein, 10 aa, synthetic construct
  REGION 1..10: note = Affinity peptide
FGRLVSSIRY

SEQ ID NO: 30 - protein, 10 aa, synthetic construct
  REGION 1..10: note = Affinity peptide
TWKTSRISIF

SEQ ID NO: 31 - protein, 4 aa, synthetic construct
  REGION 1..4: note = Affinity peptide
QSYP

SEQ ID NO: 32 - protein, 6 aa, synthetic construct
  REGION 1..6: note = Affinity peptide
HWRGWV

SEQ ID NO: 33 - protein, 6 aa, synthetic construct
  REGION 1..6: note = Affinity peptide
HYFKFD

SEQ ID NO: 34 - protein, 6 aa, synthetic construct
  REGION 1..6: note = Affinity peptide
HFRRHL

SEQ ID NO: 35 - protein, 4 aa, synthetic construct
  REGION 1..4: note = Affinity peptide
DAAG

SEQ ID NO: 36 - protein, 8 aa, synthetic construct
  REGION 1..8: note = Affinity peptide
NARKFYKG

SEQ ID NO: 37 - protein, 8 aa, synthetic construct
  REGION 1..8: note = Affinity peptide
NKFRGKYK

SEQ ID NO: 38 - protein, 17 aa, synthetic construct
  REGION 1..17: note = Affinity peptide (Fc3K).Two cysteine residues may be linked viadisulfide bridge.
RGNCAYHKGQIIWCTYH

SEQ ID NO: 39 - protein, 34 aa, synthetic construct
  REGION 1..34: note = Affinity peptide (Z34CK).Two cysteine residues may be linkedvia disulfide bridge.
FNKQCQRRFYEALHDPNLNEEQRNARIRSIREEC

SEQ ID NO: 40 - protein, 34 aa, synthetic construct
  REGION 1..34: note = Affinity peptide (Z34CM).Two cysteine residues may be linkedvia disulfide bridge.
FNMQCQRRFYEALHDPNLNEEQRNARIRSIREEC

SEQ ID NO: 41 - protein, 44 aa, synthetic construct
  REGION 1..44: note = Affinity peptide (ProAR).Two cysteine residues may be linkedvia disulfide bridge.
FNREQQNAFYEILHLPNLNEEQRNGFIQSLRDDPSQSANLLAEA

SEQ ID NO: 42 - protein, 30 aa, synthetic construct
  REGION 1..30: note = Signal peptide of caspase B (CspBss)
MFNNRIRTAALAGAIAISTAASGVAIPAFA

SEQ ID NO: 43 - DNA, 1268 bp, synthetic construct
  source 1..1268: mol_type = other DNA
ggtaccggagaccacaacggtttccctctagaaataattttgtttaactttaagaaggagatataccaatggatgagttcgagatgatcaaacgtaacacttccgagatcatttccgaggaagaactgcgcgaagtgcttaagaaagatgagaagtctgcgacgattggcttcgaaccatcagggaagattcaccttggccactacttgcagatcaagaagatgatcgacttgcagaatgctggcttcgacatcatcattctgctggcggatctgcatgcctacctcaatcagaagggagaactggacgaaatccgcaagatcggcgactacaacaagaaagtctttgaagcaatgggtctgaaggcgaaatacgtctatgggagcaacttccagcttgacaaagactacaccttgaacgtgtatcggcttgctctgaaaaccacactcaaacgtgcacgccgatcgatggaactcatcgcacgggaggacgagaatccgaaggttgctgaagtcatctatcccatcatgcaagttaacccgcttcattaccaaggagtggatgttgcagttggtggtatggaacagcgcaagattcacatgttggcacgcgaactgctgccgaagaaagtggtctgcatccacaatcccgtgctcactggtttggacggtgaaggcaagatgagctcctctaaaggcaactttatcgctgtcgatgattcgcctgaagagattcgtgccaagattaagaaggcttactgtccagcgggagtagtggaaggcaacccaatcatggagattgccaagtacttcctggagtatccattgaccatcaagcgtcctgagaagtttggcggtgatctcaccgtaaactcctacgaggaactggaatccctcttcaagaacaaagagctgcacccaatggatctcaagaacgcagttgccgaggagctgatcaagatccttgagcctattcgcaaacgcctgtaagggcccggcatggatgaactatacgatctactcgttactcaaggcaagctcgagcgggacggtcgaaccagcttcaagcgaccggatgagtatgttacagtagatagcgacggggtctcatagtaaagtatgaggcgcaccaaacgaggtgccccccgccttagttcagcagggcagaacggcggactctaaatccgcatggcacgggttcaaatcccgtaggcgggaccactgcagatccttagcgaaagctaaggatttttttttgatatctctaga

SEQ ID NO: 44 - DNA, 921 bp, synthetic construct
  source 1..921: mol_type = other DNA
atggatgagttcgagatgatcaaacgtaacacttccgagatcatttccgaggaagaactgcgcgaagtgcttaagaaagatgagaagtctgcgacgattggcttcgaaccatcagggaagattcaccttggccactacttgcagatcaagaagatgatcgacttgcagaatgctggcttcgacatcatcattctgctggcggatctgcatgcctacctcaatcagaagggagaactggacgaaatccgcaagatcggcgactacaacaagaaagtctttgaagcaatgggtctgaaggcgaaatacgtctatgggagcaacttccagcttgacaaagactacaccttgaacgtgtatcggcttgctctgaaaaccacactcaaacgtgcacgccgatcgatggaactcatcgcacgggaggacgagaatccgaaggttgctgaagtcatctatcccatcatgcaagttaacccgcttcattaccaaggagtggatgttgcagttggtggtatggaacagcgcaagattcacatgttggcacgcgaactgctgccgaagaaagtggtctgcatccacaatcccgtgctcactggtttggacggtgaaggcaagatgagctcctctaaaggcaactttatcgctgtcgatgattcgcctgaagagattcgtgccaagattaagaaggcttactgtccagcgggagtagtggaaggcaacccaatcatggagattgccaagtacttcctggagtatccattgaccatcaagcgtcctgagaagtttggcggtgatctcaccgtaaactcctacgaggaactggaatccctcttcaagaacaaagagctgcacccaatggatctcaagaacgcagttgccgaggagctgatcaagatccttgagcctattcgcaaacgcctgtaa

SEQ ID NO: 45 - protein, 306 aa, Methanococcus jannaschii
MDEFEMIKRNTSEIISEEELREVLKKDEKSATIGFEPSGKIHLGHYLQIKKMIDLQNAGFDIIILLADLHAYLNQKGELDEIRKIGDYNKKVFEAMGLKAKYVYGSNFQLDKDYTLNVYRLALKTTLKRARRSMELIAREDENPKVAEVIYPIMQVNPLHYQGVDVAVGGMEQRKIHMLARELLPKKVVCIHNPVLTGLDGEGKMSSSKGNFIAVDDSPEEIRAKIKKAYCPAGVVEGNPIMEIAKYFLEYPLTIKRPEKFGGDLTVNSYEELESLFKNKELHPMDLKNAVAEELIKILEPIRKRL

SEQ ID NO: 46 - DNA, 77 bp, Methanococcus jannaschii
  source 1..77: mol_type = other DNA
cccgccttagttcagcagggcagaacggcggactctaaatccgcatggcacgggttcaaatcccgtaggcgggacca

SEQ ID NO: 47 - RNA, 77 nt, Methanococcus jannaschii
  source 1..77: mol_type = tRNA
cccgccttagttcagcagggcagaacggcggactctaaatccgcatggcacgggttcaaatcccgtaggcgggacca

SEQ ID NO: 48 - protein, 159 aa, synthetic construct
QVQLQESGGGLVQAGGSLRLSCAASGRTFSNYHMGWFRQAPGKERELVAAISGSGGSTYYTDSVKGRFTISRNNAKNTMSLQMSNLKPEDTGVYYCTTPTEKGSSIDYWGQGTQVTVSSGRYPYDVPDYAAPAAPAPAAPAAPAPAAPAAPAPHHHHHH

SEQ ID NO: 49 - protein, 160 aa, synthetic construct
QVQLQESGGGLVQAGGSLRLSCAASGRTFSNYHMGWFRQAPGKERELVAAISGSGGSTYYTDSVKGRFTISRNNAKNTMSLQMSNLKPEDTGVYYCTTPTEKGSSIDYWGQGTQVTVSSGRYPYDVPDYAAPAAPAPAAPAFAPAPAAPAAPAPHHHHHH

SEQ ID NO: 50 - DNA, 555 bp, synthetic construct
  source 1..555: mol_type = other DNA
atgaaacgcatgaaatcgctggctgcggcgctcaccgtcgctggggccatgctggccgcacctgtggcaacggcacaggtacagctacaggaatccggaggcggtcttgtacaggcaggaggcagtttgcgtctgtcctgtgctgcgtctggtcgtacgttctccaactatcacatggggtggtttcgccaagcaccaggcaaagaacgcgagttggttgccgccattagcgggtctggaggaagcacgtactacaccgatagcgtcaaaggccgtttcacgatcagccgcaataacgctaagaacaccatgtctctgcagatgtcgaacctcaagcctgaagacactggcgtgtactactgcactacacctaccgagaaaggttcctcgatcgactattggggtcaaggcactcaagtcaccgtctcgagtgggaggtatccctatgatgtgccggattatgctgcacccgcagcacccgcgccagcagcgccagctgcgcctgctccagcagcaccagccgctcctgctccgcaccatcaccaccatcactaa

SEQ ID NO: 51 - protein, 184 aa, synthetic construct
MKRMKSLAAALTVAGAMLAAPVATAQVQLQESGGGLVQAGGSLRLSCAASGRTFSNYHMGWFRQAPGKERELVAAISGSGGSTYYTDSVKGRFTISRNNAKNTMSLQMSNLKPEDTGVYYCTTPTEKGSSIDYWGQGTQVTVSSGRYPYDVPDYAAPAAPAPAAPAAPAPAAPAAPAPHHHHHH

SEQ ID NO: 52 - DNA, 558 bp, synthetic construct
  source 1..558: mol_type = other DNA
atgaaacgcatgaaatcgctggctgcggcgctcaccgtcgctggggccatgctggccgcacctgtggcaacggcacaggtacagctacaggaatccggaggcggtcttgtacaggcaggaggcagtttgcgtctgtcctgtgctgcgtctggtcgtacgttctccaactatcacatggggtggtttcgccaagcaccaggcaaagaacgcgagttggttgccgccattagcgggtctggaggaagcacgtactacaccgatagcgtcaaaggccgtttcacgatcagccgcaataacgctaagaacaccatgtctctgcagatgtcgaacctcaagcctgaagacactggcgtgtactactgcactacacctaccgagaaaggttcctcgatcgactattggggtcaaggcactcaagtcaccgtctcgagtgggaggtatccctatgatgtgccggattatgctgcacccgcagcacccgcgccagcagcgccagcttaggcgcctgctccagcagcaccagccgctcctgctccgcaccatcaccaccatcactaa

SEQ ID NO: 53 - protein, 184 aa, synthetic construct
MKRMKSLAAALTVAGAMLAAPVATAQVQLQESGGGLVQAGGSLRLSCAASGRTFSNYHMGWFRQAPGKERELVAAISGSGGSTYYTDSVKGRFTISRNNAKNTMSLQMSNLKPEDTGVYYCTTPTEKGSSIDYWGQGTQVTVSSGRYPYDVPDYAAPAAPAPAAPAFAPAPAAPAAPAPHHHHH

SEQ ID NO: 54 - protein, 102 aa, synthetic construct
QETRGNCAYHKGQIIWCTYHGGGGSGGAAPAAPAPAAPAAPAPAAPAAPAPAAPAAPAPAAPAAPAPAAPAAPAPGGSGGGGSGGRGNCAYHRGQIIWCTYH

SEQ ID NO: 55 - protein, 99 aa, synthetic construct
QETRGNCAYHKGQIIWCTYHGGGAAPASPAPAAPASPAPAAPASPAPAAPASPAPAAPASPAPAAPASPAPAAPASPAPGGGRGNCAYHRGQIIWCTYH

SEQ ID NO: 56 - protein, 101 aa, synthetic construct
QETRGNCAYHKGQIIWCTYHGGAPSSPSPSAPSSPSPASPSSAPSSPSPSAPSSPSPASPSSAPSSPSPSAPSSPSPASPSSGGRGNCAYHRGQIIWCTYH

SEQ ID NO: 57 - protein, 105 aa, synthetic construct
QETRGNCAYHKGQIIWCTYHGGASPSAPAPASPSAPAPASPSAPAPASPSAPAPASPSAPAPASPSAPAPASPSAPAPASPSAPAPGGRGNCAYHRGQIIWCTYH

SEQ ID NO: 58 - protein, 109 aa, synthetic construct
QETRGNCAYHKGQIIWCTYHGGAPSSPSPSAPSSPSPASPSSPAPAPAPAPAPAPAPAPAPAPAPAPAPAAPSSPSPSAPSSPSPASPSSGGRGNCAYHRGQIIWCTYH

SEQ ID NO: 59 - protein, 121 aa, synthetic construct
QETRGNCAYHKGQIIWCTYHGGAPSSPSPSAPSSPSPASPSSAPSSPSPSAPSSPSPASPSSAPSSPSPSAPSSPSPASPSSAPSSPSPSAPSSPSPASPSSGGRGNCAYHRGQIIWCTYH

SEQ ID NO: 60 - DNA, 399 bp, synthetic construct
  source 1..399: mol_type = other DNA
atgtttaacaaccgtatccgcactgcagctctcgctggtgcaatcgcaatctccaccgcagcttccggcgtagctatcccagcattcgctcaggagacccgtggcaattgcgcctatcacaagggtcagatcatttggtgcacctaccatggtggtggaggttctggtggtgccgccccggctgcaccagcgccagcggccccagcggctcctgcaccggctgctccagctgcgccagctcctgcagctcccgcagcaccggcgcctgcagcaccagcggcaccagcacccgccgctccggccgcccctgcccccggcggctccgggggaggcggcagcggaggacgcggtaactgcgcataccatcgcggccaaattatctggtgcacttatcactaa

SEQ ID NO: 61 - protein, 132 aa, synthetic construct
MFNNRIRTAALAGAIAISTAASGVAIPAFAQETRGNCAYHKGQIIWCTYHGGGGSGGAAPAAPAPAAPAAPAPAAPAAPAPAAPAAPAPAAPAAPAPAAPAAPAPGGSGGGGSGGRGNCAYHRGQIIWCTYH

SEQ ID NO: 62 - DNA, 390 bp, synthetic construct
  source 1..390: mol_type = other DNA
atgtttaacaaccgtatccgcactgcagctctcgctggtgcaatcgcaatctccaccgcagcttccggcgtagctatcccagcattcgctcaggagacccgtggcaattgcgcctatcacaagggtcagatcatttggtgcacctaccatggtggtggtgccgctccagcatccccagccccggccgcacctgcaagccctgctcccgctgctccggcttcaccagcgccagcagcacctgcctctcccgctcctgcggcaccagcgagtcctgcgccagccgctccggcatcgcccgcaccagcggctccggcctccccggcccccggcggaggacgcggtaactgcgcataccatcgcggccaaattatctggtgcacttatcactaa

SEQ ID NO: 63 - protein, 129 aa, synthetic construct
MFNNRIRTAALAGAIAISTAASGVAIPAFAQETRGNCAYHKGQIIWCTYHGGGAAPASPAPAAPASPAPAAPASPAPAAPASPAPAAPASPAPAAPASPAPAAPASPAPGGGRGNCAYHRGQIIWCTYH

SEQ ID NO: 64 - DNA, 396 bp, synthetic construct
  source 1..396: mol_type = other DNA
atgtttaacaaccgtatccgcactgcagctctcgctggtgcaatcgcaatctccaccgcagcttccggcgtagctatcccagcattcgctcaggagacccgtggcaattgcgcctatcacaagggtcagatcatttggtgcacctaccatggtggtgccccatcctctccctcaccctcggcaccgagctccccatctccggcgtcaccatcctccgcaccctcttccccttctccatcggctccttcgtccccttccccagcttcccctagctccgcaccgtccagcccctctccatcagcgccttcctcgccatcaccggcctctccgagctccggaggacgcggtaactgcgcataccatcgcggccaaattatctggtgcacttatcactaa

SEQ ID NO: 65 - protein, 131 aa, synthetic construct
MFNNRIRTAALAGAIAISTAASGVAIPAFAQETRGNCAYHKGQIIWCTYHGGAPSSPSPSAPSSPSPASPSSAPSSPSPSAPSSPSPASPSSAPSSPSPSAPSSPSPASPSSGGRGNCAYHRGQIIWCTYH

SEQ ID NO: 66 - DNA, 408 bp, synthetic construct
  source 1..408: mol_type = other DNA
atgtttaacaaccgtatccgcactgcagctctcgctggtgcaatcgcaatctccaccgcagcttccggcgtagctatcccagcattcgctcaggagacccgtggcaattgcgcctatcacaagggtcagatcatttggtgcacctaccatggtggtgcgtccccctcagctcccgcacctgcgagtcctagcgcgccagcacctgcatccccttccgctccggcacctgcctctccgtcagcaccggctccagcaagcccatccgccccagctccagcttctccgtccgcaccagcccccgcctctccttcggcgccagctccggcgtcgccaagcgctccagcccccggaggacgcggtaactgcgcataccatcgcggccaaattatctggtgcacttatcactaa

SEQ ID NO: 67 - protein, 135 aa, synthetic construct
MFNNRIRTAALAGAIAISTAASGVAIPAFAQETRGNCAYHKGQIIWCTYHGGASPSAPAPASPSAPAPASPSAPAPASPSAPAPASPSAPAPASPSAPAPASPSAPAPASPSAPAPGGRGNCAYHRGQIIWCTYH

SEQ ID NO: 68 - DNA, 420 bp, synthetic construct
  source 1..420: mol_type = other DNA
atgtttaacaaccgtatccgcactgcagctctcgctggtgcaatcgcaatctccaccgcagcttccggcgtagctatcccagcattcgctcaggagacccgtggcaattgcgcctatcacaagggtcagatcatttggtgcacctaccatggtggtgcaccgagctctccctccccctctgccccgtcttcgccgtcaccagcttccccatccagtccagctccggcgcctgcccctgccccagcaccggctcctgctcctgcgccagctccagcaccagcgcctgcaccagcccctgcagcaccctcctcaccatcgccaagtgcgccctcctccccttccccggcttctcccagcagcggaggacgcggtaactgcgcataccatcgcggccaaattatctggtgcacttatcactaa

SEQ ID NO: 69 - protein, 139 aa, synthetic construct
MFNNRIRTAALAGAIAISTAASGVAIPAFAQETRGNCAYHKGQIIWCTYHGGAPSSPSPSAPSSPSPASPSSPAPAPAPAPAPAPAPAPAPAPAPAPAPAAPSSPSPSAPSSPSPASPSSGGRGNCAYHRGQIIWCTYH

SEQ ID NO: 70 - DNA, 456 bp, synthetic construct
  source 1..456: mol_type = other DNA
atgtttaacaaccgtatccgcactgcagctctcgctggtgcaatcgcaatctccaccgcagcttccggcgtagctatcccagcattcgctcaggagacccgtggcaattgcgcctatcacaagggtcagatcatttggtgcacctaccatggtggtgccccgtcctccccatccccatctgccccttcgagcccatcccctgcatcaccctcctcggctccttcctcaccctctccatccgcgccatctagcccatctccagcctccccttcttccgctccttcatctccttcgccctccgcacccagctccccaagccctgcgtccccgtctagcgcaccgtcgtcgccgtccccatccgcaccgtcatccccgtcaccagctagcccctcctccggaggacgcggtaactgcgcataccatcgcggccaaattatctggtgcacttatcactaa

SEQ ID NO: 71 - protein, 151 aa, synthetic construct
MFNNRIRTAALAGAIAISTAASGVAIPAFAQETRGNCAYHKGQIIWCTYHGGAPSSPSPSAPSSPSPASPSSAPSSPSPSAPSSPSPASPSSAPSSPSPSAPSSPSPASPSSAPSSPSPSAPSSPSPASPSSGGRGNCAYHRGQIIWCTYH

SEQ ID NO: 72 - DNA, 1563 bp, synthetic construct
  source 1..1563: mol_type = other DNA
gtgagccaagccctacctgttcgtgaccaggggcgggaccaggggattttcgctggtactctcccgcccgcaccgccaaagttcaagtggacccgcctggatacctatacctgggcgatcatcgcggtgtttgctttagtcacgcgttttacaggtttgagcagtgcaaccgcctcaggcaccccagtttttgatgaaaaacactacgtcccacaagcctgggacatggtccgctcctggatcaaccccatcaccggcggcattgaatccaaccccggatacggactcgtcgttcacccaccgttggccaaacaacttgaagcactcggtgaatgggtcttcggatacacccccctcggctggcgcatcatggtcgccattttcggaacactcaccattttcgccatcatggcaatcgcacggcgcctcagcggatccaccattgtgactttcatcgccggaattctcgcgcttgccgacggcgtcctcctcgtctcatcacgcttcggcatgctggacatcttccttgttttcttcatcaccgcagcagcatgggcattgatccgagatcaccaacaaatgcaccaacgcctcaacgatttactcctcaccaacggccaaatcaccaaagactttggcccccgattcggcttccgatggtggcgtttcaccacaggtgtattccttggtctcgcgctctccgtcaaatggtccggactgtactacatcgcattcttcggcctgaccagcgtgttcctagacttgtggctgcgcaaacgctacggcgtccgacgctacgtcaccggcaccctaaaaaatgacgtcatcccagcgctcggctccttggtgatcatccctgccctgctttatatctggagctggcgagcctggttcgcctccgaaacctccgtctaccgccacgccaaaacagacggcaccatcacagaagactccatcctgcagctcttccctgaatcaattgcgggctggatccactatcacatcagcgtcctggaattccacggctcactgaccacatcctcaggtcacagccacccctgggattccaagccgtgggcctggcttgtctccggtcgacccatcctctacttctcctccaccgacatctcctgcgacgttggcggcacctgccgacgcatgatctacctcttcggcacgcccgccatttggtggctgacagtcccagtcattctgtgggcgctgtggtctttcttcgcacgtcggagtcgtggctatattgtcccactagtggccttcgctgcaggatttttgccgtggcttgcagcatacgaccgccaaatgtacttcttctacgccaccgcattggtgccattcaccatcatcatgttggcactcgcctgcggtgaactgtggggccgtggaaaaatgacccccactggcttaacccgcggatcaatggcagtggtcacctacatttccctcgtggtgatgatgtttctcgcgttttcgccactgttttacggatttgtcatcccagattatgtctacgaatccttgatgtggttcccaagctggcgctaa

SEQ ID NO: 73 - protein, 520 aa, synthetic construct
MSQALPVRDQGRDQGIFAGTLPPAPPKFKWTRLDTYTWAIIAVFALVTRFTGLSSATASGTPVFDEKHYVPQAWDMVRSWINPITGGIESNPGYGLVVHPPLAKQLEALGEWVFGYTPLGWRIMVAIFGTLTIFAIMAIARRLSGSTIVTFIAGILALADGVLLVSSRFGMLDIFLVFFITAAAWALIRDHQQMHQRLNDLLLTNGQITKDFGPRFGFRWWRFTTGVFLGLALSVKWSGLYYIAFFGLTSVFLDLWLRKRYGVRRYVTGTLKNDVIPALGSLVIIPALLYIWSWRAWFASETSVYRHAKTDGTITEDSILQLFPESIAGWIHYHISVLEFHGSLTTSSGHSHPWDSKPWAWLVSGRPILYFSSTDISCDVGGTCRRMIYLFGTPAIWWLTVPVILWALWSFFARRSRGYIVPLVAFAAGFLPWLAAYDRQMYFFYATALVPFTIIMLALACGELWGRGKMTPTGLTRGSMAVVTYISLVVMMFLAFSPLFYGFVIPDYVYESLMWFPSWR

SEQ ID NO: 74 - DNA, 26 bp, synthetic construct
  source 1..26: mol_type = other DNA
gtttcgtacctaaaccgacccgaacc

SEQ ID NO: 75 - DNA, 24 bp, synthetic construct
  source 1..24: mol_type = other DNA
tcggttgattgtagagccttggcg

SEQ ID NO: 76 - DNA, 46 bp, synthetic construct
  source 1..46: mol_type = other DNA
gccaaggctctacaatcaaccgatggccgaaccaagtgaccaatgc

SEQ ID NO: 77 - DNA, 25 bp, synthetic construct
  source 1..25: mol_type = other DNA
aagctccggcattgattccgttacc

SEQ ID NO: 78 - protein, 17 aa, synthetic construct
RGNCAYHRGQIIWCTYH

SEQ ID NO: 79 - protein, 18 aa, synthetic construct
RGNCAYHKGQIIWCTYHF